European Patent Application EP 4 779 019 A2, published July 22, 2026. Title: TARGETING NRIP1 TO ALLEVIATE METABOLIC DISEASE. Applicant: University of Massachusetts. Application IB PCT/US2021/054155, filed October 8, 2021. The sequence listing filed with the application follows.

SEQUENCE LISTING (44 sequences)

SEQ ID NO: 1 - protein, 7 aa, synthetic construct
  REGION 1..7: note = SV40 large T antigen NLS
PKKKRRV

SEQ ID NO: 2 - protein, 7 aa, synthetic construct
  REGION 1..7: note = SV40 large T antigen NLS
PKKKRKV

SEQ ID NO: 3 - protein, 18 aa, synthetic construct
  REGION 1..18: note = SV40 large T antigen NLS
KRTADGSEFESPKKKRKV

SEQ ID NO: 4 - protein, 16 aa, synthetic construct
  REGION 1..16: note = nucleoplasmin NLS
KRPAATKKAGQAKKKK

SEQ ID NO: 5 - DNA, 60 bp, synthetic construct
  misc_feature 1..60: note = polyadenylation signal
  source 1..60: mol_type = other DNA
tagcaataaaggatcgtttattttcattggaagcgtgtgttggttttttgatcaggcgcg

SEQ ID NO: 6 - RNA, 20 nt, Mus musculus
  source 1..20: mol_type = other RNA
cttgtattgaacatgactca

SEQ ID NO: 7 - RNA, 20 nt, Mus musculus
  source 1..20: mol_type = other RNA
attgtcttaacttacctcga

SEQ ID NO: 8 - RNA, 20 nt, Mus musculus
  source 1..20: mol_type = other RNA
gtcagtacccagacgtacca

SEQ ID NO: 9 - RNA, 20 nt, Mus musculus
  source 1..20: mol_type = other RNA
ataaggtttggagtcacgtc

SEQ ID NO: 10 - RNA, 20 nt, Mus musculus
  source 1..20: mol_type = other RNA
cactttgtcccactgcggga

SEQ ID NO: 11 - RNA, 20 nt, Mus musculus
  source 1..20: mol_type = other RNA
acaggctgttgccagcatgg

SEQ ID NO: 12 - RNA, 20 nt, Mus musculus
  source 1..20: mol_type = other RNA
ggagtcgaagaacatctgca

SEQ ID NO: 13 - RNA, 20 nt, Homo sapiens
  source 1..20: mol_type = other RNA
cttctattgaacatgactca

SEQ ID NO: 14 - RNA, 20 nt, Homo sapiens
  source 1..20: mol_type = other RNA
gcttggctctgatgtgcacc

SEQ ID NO: 15 - RNA, 20 nt, Homo sapiens
  source 1..20: mol_type = other RNA
acacatacatatcaggggtc

SEQ ID NO: 16 - RNA, 20 nt, Homo sapiens
  source 1..20: mol_type = other RNA
acatcaggaagattcgtatc

SEQ ID NO: 17 - RNA, 20 nt, Homo sapiens
  source 1..20: mol_type = other RNA
gtcatgtgctgcaagattac

SEQ ID NO: 18 - RNA, 20 nt, Homo sapiens
  source 1..20: mol_type = other RNA
tttgcatggtccctaagaaa

SEQ ID NO: 19 - RNA, 20 nt, synthetic construct
  misc_feature 1..20: note = Non-Targeting control sgRNA
  source 1..20: mol_type = other RNA
gcactaccagagctaactca

SEQ ID NO: 20 - DNA, 4153 bp, Mus musculus
  source 1..4153: mol_type = other DNA
tactgacgtgcgtttggtgagcaacgaaagatgatgaagaaagaaaaccagcatattccctgagacctgggtgccagcgctgccgctgtgctaaggaagttgcgaggctggcccttgcctagccactcatcagtgctgtagtctgcacccgagtttgccccagcctctgagcccctcgtcactgcctgaagatcccctggtcagaatgttaacagtgcatctctgcccgactgctatgggaggtgatcaggtgacgctcacttcctgacgtcacgtgggatcttactgacgagaggagctctttcacgtgaacggaagccgagcccctgtgagcgcttgtattgaacatgactcatggagaagagcttggctctgatgtgcatcaggattctattgtcttaacttacctcgaagggttactaatgcatcaggcagcagggggatcaggcactgccattaacaaaaagtctgctggccacaaagaggaagaccagaactttaacctctcgggcagtgcgtttccctcctgtcaaagcaatggtcccactgtcagtacccagacgtaccagggatctggcatgctgcacctcaaaaaagccagactgctgcagtcttccgaggactggaacgcggcaaagcggaagaggctgtctgattccatcgtgaatttaaacgtaaagaaggaagcgttgctggctggcatggttgacagtgtgcctaaaggcaaacaggatagcacattgctggcctctttgcttcagtcattcagctctaggctgcagactgttgctctgtcacagcagattagacagagcctcaaggagcagggatatgccctcagtcacgagtctttaaaagtggagaaggatttaaggtgctatggcgtggcctcaagtcacttaaaaactctgttgaagaaaagtaaaaccaaggatcaaaagtcaggtcccaccctccctgacgtgactccaaaccttatcagagatagctttgttgagtcatcccatcccgcagtgggacaaagtgggacaaaggtcatgagtgagcccttgtcatgtgctgcaagattacaggctgttgccagcatggtggagaaaagggcgagtcccgctgcctccccaaagcctagtgttgcctgcagccagttggcgctgctcctgtccagcgaggcccacctgcagcagtactctcgggaacatgctctaaaaacgcagaacgcacatcaggtggcaagcgaaagacttgcagccatggccagattgcaagagaatgggcagaaggacgtgggcagttcgcagctctccaaaggggtgtctggccatctcaacgggcaggccagagcactgccggcaagcaaactggtggccaacaagaataacgctgccacctttcagagtccaatgggtgttgtcccttcctcccccaaaaacacgagctataagaactcactggaaagaaacaacctaaagcaggctgctaataacagtctgcttttgcatctcctcaaaagccagaccatacccacgccgatgaacgggcacagccagaacgagagagcgagcagttttgagagtagcacgcccaccacgattgatgagtactccgataacaacccgagctttacagatgacagcagtggagacgaaagctcgtactccaattgcgttcccatagacctgtcttgcaaacaccggatcgaaaagccggaagctgagcggcccgtttcgctggagaacctaacccagtccttgttaaacacgtgggatcccaagatccccggcgttgacatcaaagaagatcaagatacctcaacaaattccaagctgaattcacaccagaaagtcactcttcttcagttgctgctcggccataaaagtgaagaaactgttgaaaggaacgccagccctcaggacatccatagtgatgggactaagttcagtcctcagaattacacaaggacttctgtcatcgaaagccccagtaccaacaggactaccccagtgagcactccaccactgtatacagccagccaagcagagtctcccatcaatctttcccagcactctctggtcatcaagtggaattccccgccgtatgcctgcagtactcccgcttccaagctcacgaacaccgcgcctagccacctgatggacctcacgaaaggcaaagagtcccaagccgagaaaccagccccgagtgaaggtgcacaaaattccgccacgttcagtgccagtaaactgttacaaaatttggctcagtgcggattgcagtcttccgggccaggggaagagcagagaccctgcaaacagctgttaagtggaaacccagacaaacctctcggtctgattgatagattaaacagccctctgctctcaaataaaaccaatgcggctgaagagagcaaagccttcagcagtcagcctgccgggcctgagccgggacttcctggttgtgagatagaaaatctcttggaaagacggactgtccttcagttgctcctgggaaattccagcaaagggaagaatgagaagaaagagaaaacccccgcacgagacgaggctcctcaggagcattcggagagggctgcaaatgaacagatactcatggtgaagattaaatccgagccttgtgacgacttccagacccacaacacaaacctgcccttaaaccacgatgccaagagcgcccccttcttaggtgtgactcccgccatccacaggagcacagcggccttaccagtgtcggaggactttaaatccgagcctgcttcacctcaggatttctctttctcaaagaacgggctgttgagtcgcttgctgagacagaatcaagagagttacccggcagatgagcaggacaagagtcacagaaacagtgagctgccaaccctggagtcgaagaacatctgcatggtcccgaagaaaaggaagctgtatacggaaccactggagaatccatttaaaaagatgaaaaatactgccgtagatactgccaatcatcacagcggcccggaagtactctacgggtcgttgcttcatcaggaagagctgaagtttagcaggaatgagctcgattataaataccctgctgggcatagttcagccagcgatggtgaccacaggagttgggccagagagagcaaaagcttcaatgttctcaagcagctgctgctctccgagaactgtgtgcgagatctgtccccacacaggagtgactctgtccccgacacgaaaaagaaaggacacaaaaacaacgcgcccggcagcaaacctgaattcggcatttcttctttaaatggactgatgtatagttccccgcagcctggcagttgtgtgacggatcataggacattttcatacccgggaatggtaaagacccctctgagccctcctttcccagagcacttgggctgtgtggggtccagaccagaacctgggcttttgaatggatgttccgtgcccggtgagaagggacccattaagtgggtcatcgcagatatggataagaatgaatacgaaaaagactctccaagactgaccaaaactaatccgatcctctattacatgctccagaagggagggggcaattctgttaccacacaagaaacccaggacaaagacatctggagggagcctgcgtcagccgagagtctctcacaggttacagtcaaagaagagctacttcccgctgcagaaactaaagcttctttctttaatctaagaagcccgtacaatagccatatgggaaataatgcttctcgcccacacagtacaaatggagaagtgtatggacttctgggaaacgcgctcaccataaaaaaagagtcagaataaatgtgtacctgccataccactttgggtctttttaaaatttagtcagtatgaacttgagatctgtataaataagagcatgatttgagaaaagcatggtataactgaaactccttccttttgaaagtattggtcactggtgatgtttaaatatgcatactaatttttgcttaacattagatgtcatgaggaaacaattgaactcgaggttggttgtttactatttctgtatgcatcagataacaactgtgactagcctacgaatgaacctgtttttataatcgtaaataagaggcatacattaaaatgcacaacttcaccag

SEQ ID NO: 21 - DNA, 7291 bp, Homo sapiens
  source 1..7291: mol_type = other DNA
acactgatatttgcatttaatggggaacaaaagatgaagaaggaaaaggaatatattcactaaggattctatctgcttactgctacagacctatgtgttaaggaattcttctcctcctccttgcgtagaagttgatcagcactgtggtcagactgcatttatcttgtcattgccagaagaaatcttggacagaatgtaacagtacgtctctctctgattgcgatggaaggtgataaactgatactcctttattaaagttacatcgcactcaccacagaaaaccattctttaaagtgaatagaaaccaagcccttgtgaacacttctattgaacatgactcatggagaagagcttggctctgatgtgcaccaggattctattgttttaacttacctagaaggattactaatgcatcaggcagcagggggatcaggtactgccgttgacaaaaagtctgctgggcataatgaagaggatcagaactttaacatttctggcagtgcatttcccacctgtcaaagtaatggtccagttctcaatacacatacatatcaggggtctggcatgctgcacctcaaaaaagccagactgttgcagtcttctgaggactggaatgcagcaaagcggaagaggctgtctgattctatcatgaatttaaacgtaaagaaggaagctttgctagctggcatggttgacagtgtgcctaaaggcaaacaggatagcacattactggcctctttgcttcagtcattcagctctaggctgcagactgttgctctgtcacaacaaatcaggcagagcctcaaggagcaaggatatgccctcagtcatgattctttaaaagtggagaaggatttaaggtgctatggtgttgcatcaagtcacttaaaaactttgttgaagaaaagtaaagttaaagatcaaaagcctgatacgaatcttcctgatgtgactaaaaacctcatcagagataggtttgcagagtctcctcatcatgttggacaaagtggaacaaaggtcatgagtgaaccgttgtcatgtgctgcaagattacaggctgttgcaagcatggtggaaaaaagggctagtcctgccacctcacctaaacctagtgttgcttgtagccagttagcattacttctgtcaagcgaagcccatttgcagcagtattctcgagaacacgctttaaaaacgcaaaatgcaaatcaagcagcaagtgaaagacttgctgctatggccagattgcaagaaaatggccagaaggatgttggcagttaccagctcccaaaaggaatgtcaagccatcttaatggtcaggcaagaacatcatcaagcaaactgatggctagcaaaagtagtgctacagtgtttcaaaatccaatgggtatcattccttcttcccctaaaaatgcaggttataagaactcactggaaagaaacaatataaaacaagctgctaacaatagtttgcttttacatcttcttaaaagccagactatacctaagccaatgaatggacacagtcacagtgagagaggaagcatttttgaggaaagtagtacacctacaactattgatgaatattcagataacaatcctagttttacagatgacagcagtggtgatgaaagttcttattccaactgtgttcccatagacttgtcttgcaaacaccgaactgaaaaatcagaatctgaccaacctgtttccctggataacttcactcaatccttgctaaacacttgggatccaaaagtcccagatgtagatatcaaagaagatcaagatacctcaaagaattctaagctaaactcacaccagaaagtaacacttcttcaattgctacttggccataagaatgaagaaaatgtagaaaaaaacaccagccctcagggagtacacaatgatgtgagcaagttcaatacacaaaattatgcaaggacttctgtgatagaaagccccagtacaaatcggactactccagtgagcactccacctttacttacatcaagcaaagcagggtctcccatcaatctctctcaacactctctggtcatcaaatggaattccccaccatatgtctgcagtactcagtctgaaaagctaacaaatactgcatctaaccactcaatggaccttacaaaaagcaaagacccaccaggagagaaaccagcccaaaatgaaggtgcacagaactctgcaacgtttagtgccagtaagctgttacaaaatttagcacaatgtggaatgcagtcatccatgtcagtggaagagcagagacccagcaaacagctgttaactggaaacacagataaaccgataggtatgattgatagattaaatagccctttgctctcaaataaaacaaatgcagttgaagaaaataaagcatttagtagtcaaccaacaggtcctgaaccagggctttctggttctgaaatagaaaatctgcttgaaagacgtactgtcctccagttgctcctggggaaccccaacaaagggaagagtgaaaaaaaagagaaaactcccttaagagatgaaagtactcaggaacactcagagagagctttaagtgaacaaatactgatggtgaaaataaaatctgagccttgtgatgacttacaaattcctaacacaaatgtgcacttgagccatgatgctaagagtgccccattcttgggtatggctcctgctgtgcagagaagcgcacctgccttaccagtgtccgaagactttaaatcggagcctgtttcacctcaggatttttctttctccaagaatggtctgctaagtcgattgctaagacaaaatcaagatagttacctggcagatgattcagacaggagtcacagaaataatgaaatggcacttctagaatcaaagaatctttgcatggtccctaagaaaaggaagctttatactgagccattagaaaatccatttaaaaagatgaaaaacaacattgttgatgctgcaaacaatcacagtgccccagaagtactgtatgggtccttgcttaaccaggaagagctgaaatttagcagaaatgatcttgaatttaaatatcctgctggtcatggctcagccagcgaaagtgaacacaggagttgggccagagagagcaaaagctttaatgttctgaaacagctgcttctctcagaaaactgtgtgcgagatttgtccccgcacagaagtaactctgtggctgacagtaaaaagaaaggacacaaaaataatgtgaccaacagcaaacctgaatttagcatttcttctttaaatggactgatgtacagttccactcagcccagcagttgcatggataacaggacattttcatacccaggtgtagtaaaaactcctgtgagtcctactttccctgagcacttgggctgtgcagggtctagaccagaatctgggcttttgaatgggtgttccatgcccagtgagaaaggacccattaagtgggttatcactgatgcggagaagaatgagtatgaaaaagactctccaagattgaccaaaaccaacccaatactatattacatgcttcaaaaaggaggcaattctgttaccagtcgagaaacacaagacaaggacatttggagggaggcttcatctgctgaaagtgtctcacaggtcacagccaaagaagagttacttcctactgcagaaacgaaagcttctttctttaatttaagaagcccttacaatagccatatgggaaataatgcttctcgcccacacagcgcaaatggagaagtttatggacttctgggaagcgtgctaacgataaagaaagaatcagaataaaatgtacctgccatccagttttggatctttttaaaactaatgagtatgaacttgagatctgtataaataagagcatgatttgaaaaaaagcatggtataattgaaacttttttcattttgaaaagtattggttactggtgatgttgaaatatgcatactaatttttgcttaacattagatgtcatgaggaaactactgaactagcaattggttgtttaacacttctgtatgcatcagataacaactgtgagtagcctatgaatgaaattcttttataaatattaggcataaattaaaatgtaaaactccattcatagtggattaatgcattttgctgcctttattagggtactttattttgcttttcagaagtcagcctacataacacatttttaaagtctaaactgttaaacaactctttaaaggataattatccaataaaaaaaaacctagtgctgattcacagcttattatccaattcaaaaataaattagaaaaatatatgcttacatttttcacttttgctaaaaagaaaaaaaaaaggtgtttatttttaactcttggaagaggttttgtggttcccaatgtgtctgtcccaccctgatccttttcaatatatatttctttaaaccttgtgctacttagtaaaaattgattacaattgagggaagtttgatagatcctttaaaaaaaaggcagatttccattttttgtattttaactactttactaaattaatactcctccttttacagaattagaaaagttaacatttatctttaggtggtttcctgaaaagttgaatatttaagaaattgtttttaacagaagcaaaatggcttttctttggacagttttcaccatctcttgtaaaagttaattctcaccattcctgtggtacctgcgagtgttatgaccaggattccttaaacctgaactcagaccacttgcattagaaccatctggagcacttgttttaaaatgcagattcataggcagcatctcagatctacagaacaagaatctctgctaagtggacctggaatcttccatctgcatcttaacatgctctctaggtgtttcttgtgtttgagaaccatgacttatgactttcctcagaacatgagactgtaaaacaaaaacaaaaaactatgtgatgcctctattttccccaatacagtcacacatcagctcaaaatttgcaatattgtagttcatatattaccgttatgtctttggaaatcgggttcagaacactttttatgacaaaaattgggtggaggggataactttcatatctggctcaacatctcaggaaaatctgtgattatttgtgtgttctaatgagtaacatctacttagttagccttagggatggaaaaacagggccacttaccaaactcaggtgattccaggatggtttggaaacttctcctgaatgcatccttaacctttattaaaaccattgtcctaagaacaatgccaacaaagcttacaacatttagtttaaacccaagaagggcactaaactcagattgactaaataaaaagtacaaagggcacatatacgtgacagaattgtacacaatcactccattggatcttttactttaaagtagtgatgaaaagtacatgttgatactgtcttagaagaaattaatatattagtgaagccacatggggtttcagttgcgaaacaggtctgtttttatgttcagtttgtacaatccacaattcattcaccagatattttgttcttaattgtgaaccaggttagcaaatgacctatcaaaaattattctataatcactactagttaggatattgatttaaaattgttctacttgaagtggtttctaagatttttatattaaaaataggtgtgatttcctaatatgatctaaaaccctaaatggttatttttcctcagaatgatttgtaaatagctactggaaatattatacagtaataggagtgggtattatgcaacatcatggagaagtgaaggcataggcttattctgacataaaattccactggccagttgaatatattctattccatgtccatactatgacaatcttattgtcaacactatataaataagcttttaaacaagtcatttttcttgatcgttgtggaaggtttggagccttagaggtatgtcagaaaaaatatgttggtattctcccttgggtagggggaaatgacctttttacaagagagtgaaatttaggtcagggaaaagaccaagggccagcattgctacttttgtgtgtgtgtgtgtgggttttgttttgtttttttggttggctggttgttttcgttgttgttaacaaaggaatgagaatatgtaatacttaaataaacatgaccacgaagaatgctgttctgatttactagagaatgttcccaatttgaatttagggtgattttaaagaacagtgagaaagggcatacatccacagattcactttgtttatgcatatgtagatacaaggatgcacatatacacattttcaaggactattttagatatctagacaatttcttctaataaagtcatttgtgaaagggtactacagcttattgacatcagtaaggtagcattcattacctgtttattctctgctgcatcttacagaagagtaaactggtgagagtatatattttatatatatatatatatatatatatataatatgtatatatatatatattgacttgttacatgaagatgttaaaatcggtttttaaaggtgatgtaaatagtgatttccttaatgaaaaatacatattttgtattgttctaatgcaacagaaaagccttttaatctctttggttcctgtatattccatgtataagtgtaaatataatcagacaggtttaaaagttgtgcatgtatgtatacagttgcaagtctggacaaatgtatagaataaaccttttatttaagttgtgattacctgctgcatgaaaagtgcatgggggaccctgtgcatctgtgcatttggcaaaatgtcttaacaaatcagatcagatgttcatcctaacatgacagtattccatttctggacatgacgtctgtggtttaagctttgtgaaagaatgtgctttgattcgaagggtcttaaagaatttttttaatcgtcaaccacttttaaacataaagaattcacacaactactttcatgaattttttaatcccattgcaaacattattccaagagtatcccagtattagcaatactggaatataggcacattaccattcatagtaagaattctggtgtttacacaaccaaatttgatgcgatctgctcagtaatataatttgccatttttattagaaatttaatttcttcatgtgatgtcatgaaactgtacatactgcagtgtgaatttttttgttttgttttttaatcttttagtgtttacttcctgcagtgaatttgaataaatgagaaaaaatgcattgtc

SEQ ID NO: 22 - DNA, 20 bp, Homo sapiens
  source 1..20: mol_type = other DNA
tttgcatggtccctaagaaa

SEQ ID NO: 23 - DNA, 63 bp, synthetic construct
  misc_feature 1..63: note = synthetic nucleic acid
  source 1..63: mol_type = other DNA
ccttgtcatgtgctgcaagattacaggctgttgccagcagggggaaaaaagggggagcccccc

SEQ ID NO: 24 - DNA, 23 bp, synthetic construct
  misc_feature 1..23: note = sgRNA-M6 sequence PAM
  source 1..23: mol_type = other DNA
acaggctgttgccagcatggtgg

SEQ ID NO: 25 - DNA, 23 bp, synthetic construct
  misc_feature 1..23: note = synthetic nucleic acid
  source 1..23: mol_type = other DNA
gagggctgttgccagcatggtgg

SEQ ID NO: 26 - DNA, 23 bp, synthetic construct
  misc_feature 1..23: note = synthetic nucleic acid
  source 1..23: mol_type = other DNA
aaaggctgctgccagcatgaggg

SEQ ID NO: 27 - DNA, 23 bp, synthetic construct
  misc_feature 1..23: note = synthetic nucleic acid
  source 1..23: mol_type = other DNA
gggggctgctgccagcatggggg

SEQ ID NO: 28 - DNA, 23 bp, synthetic construct
  misc_feature 1..23: note = synthetic nucleic acid
  source 1..23: mol_type = other DNA
gtaggctgctgctagcatggtgg

SEQ ID NO: 29 - DNA, 23 bp, synthetic construct
  misc_feature 1..23: note = synthetic nucleic acid
  source 1..23: mol_type = other DNA
cacggctgctgtcagcatggtgg

SEQ ID NO: 30 - DNA, 23 bp, synthetic construct
  misc_feature 1..23: note = synthetic nucleic acid
  source 1..23: mol_type = other DNA
acaagctgttgccatcatggggg

SEQ ID NO: 31 - DNA, 23 bp, synthetic construct
  misc_feature 1..23: note = synthetic nucleic acid
  source 1..23: mol_type = other DNA
acagacagtcaccagcatggtgg

SEQ ID NO: 32 - DNA, 23 bp, synthetic construct
  misc_feature 1..23: note = synthetic nucleic acid
  source 1..23: mol_type = other DNA
acaggctgttgtcagcatgtgga

SEQ ID NO: 33 - DNA, 23 bp, synthetic construct
  misc_feature 1..23: note = synthetic nucleic acid
  source 1..23: mol_type = other DNA
aaaagctgttgccagcatgtggg

SEQ ID NO: 34 - DNA, 23 bp, synthetic construct
  misc_feature 1..23: note = synthetic nucleic acid
  source 1..23: mol_type = other DNA
ccaggctggtgccagaatggagg

SEQ ID NO: 35 - DNA, 23 bp, synthetic construct
  misc_feature 1..23: note = synthetic nucleic acid
  source 1..23: mol_type = other DNA
acaggctagggctagcatggagg

SEQ ID NO: 36 - DNA, 23 bp, synthetic construct
  misc_feature 1..23: note = synthetic nucleic acid
  source 1..23: mol_type = other DNA
acaaactgctaccagcatagtgg

SEQ ID NO: 37 - DNA, 23 bp, synthetic construct
  misc_feature 1..23: note = sgRNA-H5 sequence PAM
  misc_feature 21: note = n=a, t, c, or g
  source 1..23: mol_type = other DNA
gtcatgtgctgcaagattacngg

SEQ ID NO: 38 - DNA, 23 bp, synthetic construct
  misc_feature 1..23: note = synthetic nucleic acid
  misc_feature 21: note = n=a, t, c, or g
  source 1..23: mol_type = other DNA
atcaagttctgcaagattacngg

SEQ ID NO: 39 - DNA, 23 bp, synthetic construct
  misc_feature 1..23: note = synthetic nucleic acid
  misc_feature 21: note = n=a, t, c, or g
  source 1..23: mol_type = other DNA
gacatgtgctgaaagatttcngg

SEQ ID NO: 40 - DNA, 23 bp, synthetic construct
  misc_feature 1..23: note = synthetic nucleic acid
  misc_feature 21: note = n=a, t, c, or g
  source 1..23: mol_type = other DNA
gccatgtgctccatgattacngg

SEQ ID NO: 41 - DNA, 23 bp, synthetic construct
  misc_feature 1..23: note = synthetic nucleic acid
  misc_feature 21: note = n=a, t, c, or g
  source 1..23: mol_type = other DNA
ttcatgttctgttagattacngg

SEQ ID NO: 42 - DNA, 23 bp, synthetic construct
  misc_feature 1..23: note = synthetic nucleic acid
  misc_feature 21: note = n=a, t, c, or g
  source 1..23: mol_type = other DNA
gtcttttgctcaaagattacngg

SEQ ID NO: 43 - DNA, 899 bp, Mus musculus
  source 1..899: mol_type = other DNA
atgactcatggagaagagcttggctctgatgtgcatcaggattctattgtcttaacttacctcgaagggttactaatgcatcaggcagcagggggatcaggcactgccattaacaaaaagtctgctggccacaaagaggaagaccagaactttaacctctcgggcagtgcgtttccctcctgtcaaagcaatggtcccactgtcagtacccagacgtaccagggatctggcatgctgcacctcaaaaaagccagactgctgcagtcttccgaggactggaacgcggcaaagcggaagaggctgtctgattccatcgtgaatttaaacgtaaagaaggaagcgttgctggctggcatggttgacagtgtgcctaaaggcaaacaggatagcacattgctggcctctttgcttcagtcattcagctctaggctgcagactgttgctctgtcacagcagattagacagagcctcaaggagcagggatatgccctcagtcacgagtctttaaaagtggagaaggatttaaggtgctatggcgtggcctcaagtcacttaaaaactctgttgaagaaaagtaaaaccaaggatcaaaagtcaggtcccaccctccctgacgtgactccaaaccttatcagagatagctttgttgagtcatcccatcccgcagtgggacaaagtgggacaaaggtcatgagtgagcccttgtcatgtgctgcaagattacaggctgttgccagcatggtggagaaaagggcgagtcccgctgcctccccaaagcctagtgttgcctgcagccagttggcgctgctcctgtccagcgaggcccacctgcagcagtactctcgggaacatgctctaaaaacgcagaacgcacatcaggtggcaagcgaaagacttgc

SEQ ID NO: 44 - DNA, 896 bp, Homo sapiens
  source 1..896: mol_type = other DNA
atgactcatggagaagagcttggctctgatgtgcaccaggattctattgttttaacttacctagaaggattactaatgcatcaggcagcagggggatcaggtactgccgttgacaaaaagtctgctgggcataatgaagaggatcagaactttaacatttctggcagtgcatttcccacctgtcaaagtaatggtccagttctcaatacacatacatatcaggggtctggcatgctgcacctcaaaaaagccagactgttgcagtcttctgaggactggaatgcagcaaagcggaagaggctgtctgattctatcatgaatttaaacgtaaagaaggaagctttgctagctggcatggttgacagtgtgcctaaaggcaaacaggatagcacattactggcctctttgcttcagtcattcagctctaggctgcagactgttgctctgtcacaacaaatcaggcagagcctcaaggagcaaggatatgccctcagtcatgattctttaaaagtggagaaggatttaaggtgctatggtgttgcatcaagtcacttaaaaactttgttgaagaaaagtaaagttaaagatcaaaagcctgatacgaatcttcctgatgtgactaaaaacctcatcagagataggtttgcagagtctcctcatcatgttggacaaagtggaacaaaggtcatgagtgaaccgttgtcatgtgctgcaagattacaggctgttgcaagcatggtggaaaaaagggctagtcctgccacctcacctaaacctagtgttgcttgtagccagttagcattacttctgtcaagcgaagcccatttgcagcagtattctcgagaacacgctttaaaaacgcaaaatgcaaatcaagcagcaagtgaaagacttgc